European Patent Application EP 4 276 178 A1, published November 15, 2023. Title: Esterase Mutant and Use thereof. Applicant: ASYMCHEN LIFE SCIENCE (TIANJIN) CO., LTD. The sequence listing filed with the application follows.

SEQUENCE LISTING (2 sequences)

SEQ ID NO: 1 - protein, 314 aa, Bacillus sp. 01-855
MGSNNDNMGKRGGNLMITIPTVHKVSLPNGEVMGYRKRDGGEKTILLVHGNMTSSKHWDLFFETFPASYTLVAIDMRGFGESSYNKRVEGIEDFAQDLKFFVDQLGLNDFTMIGWSTGGAVCMQFEAQYPGYCDKIVLISSASTRGYPFFGTHSDGTPDLNQRLKTVDDIEKDPMRTIPIQQAYDTGNRALLKTIWNSLIYTHNQPEEKRYEAYVDDMMTQRNLADVYHALNTFNISSVTNGLTEGTNQANLIRIPVLVLRGERDLVISKEMTEEIVEDLGTNSTYKELSASGHSPFIDDCDQLTNIITDFLEK

SEQ ID NO: 2 - DNA, 945 bp, Bacillus sp. 01-855
atgggcagcaataacgacaacatgggtaaacgtggcggcaacctgatgatcaccatcccgacagtgcataaagtgagcctgccgaatggcgaagtgatgggttatcgtaagcgcgacggcggtgaaaaaaccatcctgctggtgcacggcaacatgaccagcagcaaacattgggacctgttcttcgagacctttccggcaagctatacactggtggccatcgatatgcgcggcttcggcgaaagcagctataacaaacgcgtggaaggcatcgaggactttgcccaggacctgaaattcttcgtggatcagctgggcctgaacgatttcaccatgatcggttggagcacaggcggcgccgtgtgtatgcagtttgaagcccagtatccgggctactgcgacaagattgtgctgattagcagcgcaagcacccgtggctatccgttttttggtacccacagcgatggcaccccggatctgaatcagcgcctgaagaccgtggacgacatcgaaaaagatcctatgcgcaccattccgatccagcaggcctacgataccggtaaccgcgccctgctgaaaaccatctggaatagcctgatttacacccacaaccagccggaggaaaagcgctatgaggcctatgtggacgacatgatgacccagcgtaatctggccgatgtgtatcacgccctgaacacattcaacattagcagcgtgaccaacggcctgaccgagggcaccaatcaggccaacctgatccgcatccctgtgctggttctgcgcggcgaacgcgacctggtgatcagcaaagagatgaccgaggagatcgtggaggatctgggcaccaacagcacctataaagagctgagcgccagcggccacagcccttttatcgatgattgcgaccagctgaccaacatcatcaccgattttctggagaaataa